European Patent Application EP 4 282 959 A1, published November 29, 2023. Title: Novel citrate synthase variant and a method for producing L-amino acid using the same. Applicant: CJ CheilJedang Corporation. The sequence listing filed with the application follows.

SEQUENCE LISTING (51 sequences)

SEQ ID NO: 1 - protein, 437 aa, Unknown
  ATCC 14067 GltA AA
MFERDIVATDNNKAVLHYPGGEFEMDIIEASEGNNGVVLGKMLSETGLITFDPGYVSTGSTESKITYIDGDAGILRYRGYDIADLAENATFNEVSYLLINGELPTPDELHKFNDEIRHHTLLDEDFKSQFNVFPRDAHPMATLASSVNILSTYYQDQLNPLDEAQLDKATVRLMAKVPMLAAYAHRARKGAPYMYPDNSLNARENFLRMMFGYPTEPYEIDPIMVKALDKLLILHADHEQNCSTSTVRMIGSAQANMFVSIAGGINALSGPLHGGANQAVLEMLEDIKNNHGGDATAFMNKVKNKEDGVRLMGFGHRVYKNYDPRAAIVKETAHEILEHLGGDDLLDLAIKLEEIALADDYFISRKLYPNVDFYTGLIYRAMGFPTDFFTVLFAIGRLPGWIAHYREQLGAAGNKINRPRQVYTGNESRKLVPREER

SEQ ID NO: 2 - DNA, 1314 bp, Unknown
  ATCC 14067 GltA NT
atgtttgaaagggatatcgtggctactgataacaacaaggctgtcctgcactaccccggtggcgagttcgaaatggacatcatcgaggcttctgagggtaacaacggtgttgtcctgggcaagatgctgtctgagactggactgatcacttttgacccaggttatgtgagcactggctccaccgagtcgaagatcacctacatcgatggcgatgcgggaatcctgcgttaccgcggctatgacatcgctgatctggctgagaatgccaccttcaacgaggtttcttacctacttatcaacggtgagctaccaaccccagatgagcttcacaagtttaacgacgagattcgccaccacacccttctggacgaggacttcaagtcccagttcaacgtgttcccacgcgacgctcacccaatggcaaccttggcttcctcggttaacattttgtctacctactaccaggatcagctgaacccactcgatgaggcacagcttgataaggcaaccgttcgcctcatggcaaaggttccaatgctggctgcgtacgcacaccgcgcacgcaagggtgctccttacatgtacccagacaactccctcaacgcgcgtgagaacttcctgcgcatgatgttcggttacccaactgagccatacgagatcgacccaatcatggtcaaggctctggacaagctgctcatcctgcacgctgaccacgagcagaactgctccacctccaccgttcgtatgatcggttccgcacaggccaacatgtttgtctccatcgctggtggcatcaacgctctgtccggcccactgcacggtggcgcaaaccaggctgttctggagatgctcgaagacatcaagaacaaccacggtggcgacgcaaccgcgttcatgaacaaggtcaagaacaaggaagacggcgtccgcctcatgggcttcggacaccgcgtttacaagaattacgatccacgtgcagcaatcgtcaaggagaccgcacacgagatcctcgagcacctcggtggcgacgatcttctggatctggcaatcaagctggaagaaattgcactggctgatgattacttcatctcccgcaagctctacccgaacgtagacttctacaccggcctgatctaccgcgcaatgggcttcccaactgacttcttcaccgtattgttcgcaatcggtcgtctgccaggatggatcgctcactaccgcgagcagctcggtgcagcaggcaacaagatcaaccgcccacgccaggtctacaccggcaacgaatcccgcaagttggttcctcgcgaggagcgctaa

SEQ ID NO: 3 - protein, 54 aa, Unknown
  ATCC 14067 GltA K415H 362~415 AA
FISRKLYPNVDFYTGLIYRAMGFPTDFFTVLFAIGRLPGWIAHYREQLGAAGNH

SEQ ID NO: 4 - protein, 437 aa, Unknown [sequence omitted]

SEQ ID NO: 5 - DNA, 1314 bp, Unknown
  ATCC13032 GltA NT
atgtttgaaagggatatcgtggctactgataacaacaaggctgtcctgcactaccccggtggcgagttcgaaatggacatcatcgaggcttctgagggtaacaacggtgttgtcctgggcaagatgctgtctgagactggactgatcacttttgacccaggttatgtgagcactggctccaccgagtcgaagatcacctacatcgatggcgatgcgggaatcctgcgttaccgcggctatgacatcgctgatctggctgagaatgccaccttcaacgaggtttcttacctacttatcaacggtgagctaccaaccccagatgagcttcacaagtttaacgacgagattcgccaccacacccttctggacgaggacttcaagtcccagttcaacgtgttcccacgcgacgctcacccaatggcaaccttggcttcctcggttaacattttgtctacctactaccaggaccagctgaacccactcgatgaggcacagcttgataaggcaaccgttcgcctcatggcaaaggttccaatgctggctgcgtacgcacaccgcgcacgcaagggtgctccttacatgtacccagacaactccctcaatgcgcgtgagaacttcctgcgcatgatgttcggttacccaaccgagccatacgagatcgacccaatcatggtcaaggctctggacaagctgctcatcctgcacgctgaccacgagcagaactgctccacctccaccgttcgtatgatcggttccgcacaggccaacatgtttgtctccatcgctggtggcatcaacgctctgtccggcccactgcacggtggcgcaaaccaggctgttctggagatgctcgaagacatcaagagcaaccacggtggcgacgcaaccgagttcatgaacaaggtcaagaacaaggaagacggcgtccgcctcatgggcttcggacaccgcgtttacaagaactacgatccacgtgcagcaatcgtcaaggagaccgcacacgagatcctcgagcacctcggtggcgacgatcttctggatctggcaatcaagctggaagaaattgcactggctgatgattacttcatctcccgcaagctctacccgaacgtagacttctacaccggcctgatctaccgcgcaatgggcttcccaactgacttcttcaccgtattgttcgcaatcggtcgtctgccaggatggatcgctcactaccgcgagcagctcggtgcagcaggcaacaagatcaaccgcccacgccaggtctacaccggcaacgaatcccgcaagttggttcctcgcgaggagcgctaa

SEQ ID NO: 6 - protein, 437 aa, Unknown
  ATCC13869 GltA AA
MFERDIVATDNNKAVLHYPGGEFEMDIIEASEGNNGVVLGKMLSETGLITFDPGYVSTGSTESKITYIDGDAGILRYRGYDIADLAENATFNEVSYLLINGELPTPDELHKFNDEIRHHTLLDEDFKSQFNVFPRDAHPMATLASSVNILSTYYQDQLNPLDEAQLDKATVRLMAKVPMLAAYAHRARKGAPYMYPDNSLNARENFLRMMFGYPTEPYEIDPIMVKALDKLLILHADHEQNCSTSTVRMIGSAQANMFVSIAGGINALSGPLHGGANQAVLEMLEDIKNNHGGDATAFMNKVKNKEDGVRLMGFGHRVYKNYDPRAAIVKETAHEILEHLGGDDLLDLAIKLEEIALADDCFISRKLYPNVDFYTGLIYRAMGFPTDFFTVLFAIGRLPGWIAHYREQLGAAGNKINRPRQVYTGKESRKLVPREER

SEQ ID NO: 7 - DNA, 1314 bp, Unknown
  ATCC13869 GltA NT
atgtttgaaagggatatcgtggctactgataacaacaaggctgtcctgcactaccccggtggcgagttcgaaatggacatcatcgaggcttctgagggtaacaacggtgttgtcctgggcaagatgctgtctgagactggactgatcacttttgacccaggttatgtgagcactggctccaccgagtcgaagatcacctacatcgatggcgatgcgggaatcctgcgttaccgcggctatgacatcgctgatctggctgagaatgccaccttcaacgaggtttcttacctacttatcaacggtgagctaccaaccccagatgagcttcacaagtttaacgacgagattcgccaccacacccttctggacgaggacttcaagtcccagttcaacgtgttcccacgcgacgctcacccaatggcaaccttggcttcctcggttaacattttgtctacctactaccaggatcagctgaacccactcgatgaggcacagcttgataaggcaaccgttcgcctcatggcaaaggttccaatgctggctgcgtacgcacaccgcgcacgcaagggtgctccttacatgtacccagacaactccctcaacgcgcgtgagaacttcctgcgcatgatgttcggttacccaaccgagccatacgagatcgacccaatcatggtcaaggctctggacaagctgctcatcctgcacgctgaccacgagcagaactgctccacctccaccgttcgtatgatcggttccgcacaggccaacatgtttgtctccatcgctggtggcatcaacgctctgtccggcccactgcacggtggcgcaaaccaggctgttctggagatgctcgaagacatcaagaacaaccacggtggcgacgcaaccgcgttcatgaacaaggtcaagaacaaggaagacggcgtccgcctcatgggcttcggacaccgcgtttacaagaactacgatccacgtgcagcaatcgtcaaggagaccgcacacgagatcctcgagcacctcggtggcgacgatcttctggatctggcaatcaagctggaagaaattgcactggctgatgattgcttcatctcccgcaagctctacccgaacgtagacttctacaccggcctgatctaccgcgcaatgggcttcccaactgacttcttcaccgtattgttcgcaatcggtcgtctgccaggatggatcgctcactaccgcgagcagctcggtgcagcaggcaacaagatcaaccgcccacgccaggtctacaccggcaaggaatcccgcaagttggttcctcgcgaggagcgctaa

SEQ ID NO: 8 - protein, 437 aa, Artificial Sequence
  ATCC 14067 GltA K415H AA
MFERDIVATDNNKAVLHYPGGEFEMDIIEASEGNNGVVLGKMLSETGLITFDPGYVSTGSTESKITYIDGDAGILRYRGYDIADLAENATFNEVSYLLINGELPTPDELHKFNDEIRHHTLLDEDFKSQFNVFPRDAHPMATLASSVNILSTYYQDQLNPLDEAQLDKATVRLMAKVPMLAAYAHRARKGAPYMYPDNSLNARENFLRMMFGYPTEPYEIDPIMVKALDKLLILHADHEQNCSTSTVRMIGSAQANMFVSIAGGINALSGPLHGGANQAVLEMLEDIKNNHGGDATAFMNKVKNKEDGVRLMGFGHRVYKNYDPRAAIVKETAHEILEHLGGDDLLDLAIKLEEIALADDYFISRKLYPNVDFYTGLIYRAMGFPTDFFTVLFAIGRLPGWIAHYREQLGAAGNHINRPRQVYTGNESRKLVPREER

SEQ ID NO: 9 - DNA, 1314 bp, Artificial Sequence
  ATCC 14067 GltA K415H NT
atgtttgaaagggatatcgtggctactgataacaacaaggctgtcctgcactaccccggtggcgagttcgaaatggacatcatcgaggcttctgagggtaacaacggtgttgtcctgggcaagatgctgtctgagactggactgatcacttttgacccaggttatgtgagcactggctccaccgagtcgaagatcacctacatcgatggcgatgcgggaatcctgcgttaccgcggctatgacatcgctgatctggctgagaatgccaccttcaacgaggtttcttacctacttatcaacggtgagctaccaaccccagatgagcttcacaagtttaacgacgagattcgccaccacacccttctggacgaggacttcaagtcccagttcaacgtgttcccacgcgacgctcacccaatggcaaccttggcttcctcggttaacattttgtctacctactaccaggatcagctgaacccactcgatgaggcacagcttgataaggcaaccgttcgcctcatggcaaaggttccaatgctggctgcgtacgcacaccgcgcacgcaagggtgctccttacatgtacccagacaactccctcaacgcgcgtgagaacttcctgcgcatgatgttcggttacccaactgagccatacgagatcgacccaatcatggtcaaggctctggacaagctgctcatcctgcacgctgaccacgagcagaactgctccacctccaccgttcgtatgatcggttccgcacaggccaacatgtttgtctccatcgctggtggcatcaacgctctgtccggcccactgcacggtggcgcaaaccaggctgttctggagatgctcgaagacatcaagaacaaccacggtggcgacgcaaccgcgttcatgaacaaggtcaagaacaaggaagacggcgtccgcctcatgggcttcggacaccgcgtttacaagaattacgatccacgtgcagcaatcgtcaaggagaccgcacacgagatcctcgagcacctcggtggcgacgatcttctggatctggcaatcaagctggaagaaattgcactggctgatgattacttcatctcccgcaagctctacccgaacgtagacttctacaccggcctgatctaccgcgcaatgggcttcccaactgacttcttcaccgtattgttcgcaatcggtcgtctgccaggatggatcgctcactaccgcgagcagctcggtgcagcaggcaaccacatcaaccgcccacgccaggtctacaccggcaacgaatcccgcaagttggttcctcgcgaggagcgctaa

SEQ ID NO: 10 - protein, 437 aa, Artificial Sequence
  ATCC13032 GltA K415H AA
MFERDIVATDNNKAVLHYPGGEFEMDIIEASEGNNGVVLGKMLSETGLITFDPGYVSTGSTESKITYIDGDAGILRYRGYDIADLAENATFNEVSYLLINGELPTPDELHKFNDEIRHHTLLDEDFKSQFNVFPRDAHPMATLASSVNILSTYYQDQLNPLDEAQLDKATVRLMAKVPMLAAYAHRARKGAPYMYPDNSLNARENFLRMMFGYPTEPYEIDPIMVKALDKLLILHADHEQNCSTSTVRMIGSAQANMFVSIAGGINALSGPLHGGANQAVLEMLEDIKSNHGGDATEFMNKVKNKEDGVRLMGFGHRVYKNYDPRAAIVKETAHEILEHLGGDDLLDLAIKLEEIALADDYFISRKLYPNVDFYTGLIYRAMGFPTDFFTVLFAIGRLPGWIAHYREQLGAAGNHINRPRQVYTGNESRKLVPREER

SEQ ID NO: 11 - DNA, 1314 bp, Artificial Sequence
  ATCC13032 GltA K415H NT
atgtttgaaagggatatcgtggctactgataacaacaaggctgtcctgcactaccccggtggcgagttcgaaatggacatcatcgaggcttctgagggtaacaacggtgttgtcctgggcaagatgctgtctgagactggactgatcacttttgacccaggttatgtgagcactggctccaccgagtcgaagatcacctacatcgatggcgatgcgggaatcctgcgttaccgcggctatgacatcgctgatctggctgagaatgccaccttcaacgaggtttcttacctacttatcaacggtgagctaccaaccccagatgagcttcacaagtttaacgacgagattcgccaccacacccttctggacgaggacttcaagtcccagttcaacgtgttcccacgcgacgctcacccaatggcaaccttggcttcctcggttaacattttgtctacctactaccaggaccagctgaacccactcgatgaggcacagcttgataaggcaaccgttcgcctcatggcaaaggttccaatgctggctgcgtacgcacaccgcgcacgcaagggtgctccttacatgtacccagacaactccctcaatgcgcgtgagaacttcctgcgcatgatgttcggttacccaaccgagccatacgagatcgacccaatcatggtcaaggctctggacaagctgctcatcctgcacgctgaccacgagcagaactgctccacctccaccgttcgtatgatcggttccgcacaggccaacatgtttgtctccatcgctggtggcatcaacgctctgtccggcccactgcacggtggcgcaaaccaggctgttctggagatgctcgaagacatcaagagcaaccacggtggcgacgcaaccgagttcatgaacaaggtcaagaacaaggaagacggcgtccgcctcatgggcttcggacaccgcgtttacaagaactacgatccacgtgcagcaatcgtcaaggagaccgcacacgagatcctcgagcacctcggtggcgacgatcttctggatctggcaatcaagctggaagaaattgcactggctgatgattacttcatctcccgcaagctctacccgaacgtagacttctacaccggcctgatctaccgcgcaatgggcttcccaactgacttcttcaccgtattgttcgcaatcggtcgtctgccaggatggatcgctcactaccgcgagcagctcggtgcagcaggcaaccacatcaaccgcccacgccaggtctacaccggcaacgaatcccgcaagttggttcctcgcgaggagcgctaa

SEQ ID NO: 12 - protein, 437 aa, Artificial Sequence
  ATCC13869 GltA K415H AA
MFERDIVATDNNKAVLHYPGGEFEMDIIEASEGNNGVVLGKMLSETGLITFDPGYVSTGSTESKITYIDGDAGILRYRGYDIADLAENATFNEVSYLLINGELPTPDELHKFNDEIRHHTLLDEDFKSQFNVFPRDAHPMATLASSVNILSTYYQDQLNPLDEAQLDKATVRLMAKVPMLAAYAHRARKGAPYMYPDNSLNARENFLRMMFGYPTEPYEIDPIMVKALDKLLILHADHEQNCSTSTVRMIGSAQANMFVSIAGGINALSGPLHGGANQAVLEMLEDIKNNHGGDATAFMNKVKNKEDGVRLMGFGHRVYKNYDPRAAIVKETAHEILEHLGGDDLLDLAIKLEEIALADDCFISRKLYPNVDFYTGLIYRAMGFPTDFFTVLFAIGRLPGWIAHYREQLGAAGNHINRPRQVYTGKESRKLVPREER

SEQ ID NO: 13 - DNA, 1314 bp, Artificial Sequence
  ATCC13869 GltA K415H NT
atgtttgaaagggatatcgtggctactgataacaacaaggctgtcctgcactaccccggtggcgagttcgaaatggacatcatcgaggcttctgagggtaacaacggtgttgtcctgggcaagatgctgtctgagactggactgatcacttttgacccaggttatgtgagcactggctccaccgagtcgaagatcacctacatcgatggcgatgcgggaatcctgcgttaccgcggctatgacatcgctgatctggctgagaatgccaccttcaacgaggtttcttacctacttatcaacggtgagctaccaaccccagatgagcttcacaagtttaacgacgagattcgccaccacacccttctggacgaggacttcaagtcccagttcaacgtgttcccacgcgacgctcacccaatggcaaccttggcttcctcggttaacattttgtctacctactaccaggatcagctgaacccactcgatgaggcacagcttgataaggcaaccgttcgcctcatggcaaaggttccaatgctggctgcgtacgcacaccgcgcacgcaagggtgctccttacatgtacccagacaactccctcaacgcgcgtgagaacttcctgcgcatgatgttcggttacccaaccgagccatacgagatcgacccaatcatggtcaaggctctggacaagctgctcatcctgcacgctgaccacgagcagaactgctccacctccaccgttcgtatgatcggttccgcacaggccaacatgtttgtctccatcgctggtggcatcaacgctctgtccggcccactgcacggtggcgcaaaccaggctgttctggagatgctcgaagacatcaagaacaaccacggtggcgacgcaaccgcgttcatgaacaaggtcaagaacaaggaagacggcgtccgcctcatgggcttcggacaccgcgtttacaagaactacgatccacgtgcagcaatcgtcaaggagaccgcacacgagatcctcgagcacctcggtggcgacgatcttctggatctggcaatcaagctggaagaaattgcactggctgatgattgcttcatctcccgcaagctctacccgaacgtagacttctacaccggcctgatctaccgcgcaatgggcttcccaactgacttcttcaccgtattgttcgcaatcggtcgtctgccaggatggatcgctcactaccgcgagcagctcggtgcagcaggcaaccacatcaaccgcccacgccaggtctacaccggcaaggaatcccgcaagttggttcctcgcgaggagcgctaa

SEQ ID NO: 14 - DNA, 5803 bp, Artificial Sequence
  pDCM2
gttcgcttgctgtccataaaaccgcccagtctagctatcgccatgtaagcccactgcaagctacctgctttctctttgcgcttgcgttttcccttgtccagatagcccagtagctgacattcatccggggtcagcaccgtttctgcggactggctttctacgtgttccgcttcctttagcagcccttgcgccctgagtgcttgcggcagcgtgaagctagcttttatcgccattcgccattcaggctgcgcaactgttgggaagggcgatcggtgcgggcctcttcgctattacgccagctggcgaaagggggatgtgctgcaaggcgattaagttgggtaacgccagggttttcccagtcacgacgttgtaaaacgacggccagtgaattcgagctcggtacccggggatcctctagagtcgacctgcaggcatgcaagcttggcgtaatcatggtcatagctgtttcctgtgtgaaattgttatccgctcacaattccacacaacatacgagccggaagcataaagtgtaaagcctggggtgcctaatgagtgagctaactcacattaattgcgttgcgctcactgcccgctttccagtcgggaaacctgtcgtgccagctgcattaatgaatcggccaacgcgcggggagaggcggtttgcgtattgggcgctcttccgcttcctcgctcactgactcgctgcgctcggtcgttcggctgcggcgagcggtatcagctcactcaaaggcggtaatacggttatccacagaatcaggggataacgcaggaaagaacatgtgagcaaaaggccagcaaaaggccaggaaccgtaaaaaggccgcgttgctggcgtttttccataggctccgcccccctgacgagcatcacaaaaatcgacgctcaagtcagaggtggcgaaacccgacaggactataaagataccaggcgtttccccctggaagctccctcgtgcgctctcctgttccgaccctgccgcttaccggatacctgtccgcctttctcccttcgggaagcgtggcgctttctcaatgctcacgctgtaggtatctcagttcggtgtaggtcgttcgctccaagctgggctgtgtgcacgaaccccccgttcagcccgaccgctgcgccttatccggtaactatcgtcttgagtccaacccggtaagacacgacttatcgccactggcagcagccactggtaacaggattagcagagcgaggtatgtaggcggtgctacagagttcttgaagtggtggcctaactacggctacactagaaggacagtatttggtatctgcgctctgctgaagccagttaccttcggaaaaagagttggtagctcttgatccggcaaacaaaccaccgctggtagcggtggtttttttgtttgcaagcagcagattacgcgcagaaaaaaaggatctcaagaagatcctttgatcttttctacggggtctgacgctcagtggaacgaaaactcacgttaagggattttggtcatgagattatcaaaaaggatcttcacctagatccttttggggtgggcgaagaactccagcatgagatccccgcgctggaggatcatccagccctgatagaaacagaagccactggagcacctcaaaaacaccatcatacactaaatcagtaagttggcagcatcacccgacgcactttgcgccgaataaatacctgtgacggaagatcacttcgcagaataaataaatcctggtgtccctgttgataccgggaagccctgggccaacttttggcgaaaatgagacgttgatcggcacgtaagaggttccaactttcaccataatgaaataagatcactaccgggcgtattttttgagttatcgagattttcaggagctgatagaaacagaagccactggagcacctcaaaaacaccatcatacactaaatcagtaagttggcagcatcacccgacgcactttgcgccgaataaatacctgtgacggaagatcacttcgcagaataaataaatcctggtgtccctgttgataccgggaagccctgggccaacttttggcgaaaatgagacgttgatcggcacgtaagaggttccaactttcaccataatgaaataagatcactaccgggcgtattttttgagttatcgagattttcaggagctctttggcatcgtctctcgcctgtcccctcagttcagtaatttcctgcatttgcctgtttccagtcggtagatattccacaaaacagcagggaagcagcgcttttccgctgcataaccctgcttcggggtcattatagcgattttttcggtatatccatcctttttcgcacgatatacaggattttgccaaagggttcgtgtagactttccttggtgtatccaacggcgtcagccgggcaggataggtgaagtaggcccacccgcgagcgggtgttccttcttcactgtcccttattcgcacctggcggtgctcaacgggaatcctgctctgcgaggctggccggctaccgccggcgtaacagatgagggcaagcggatggctgatgaaaccaagccaaccaggaagggcagcccacctatcaaggtgtactgccttccagacgaacgaagagcgattgaggaaaaggcggcggcggccggcatgagcctgtcggcctacctgctggccgtcggccagggctacaaaatcacgggcgtcgtggactatgagcacgtccgcgagggcgtcccggaaaacgattccgaagcccaacctttcatagaaggcggcggtggaatcgaaatctcgtgatggcaggttgggcgtcgcttggtcggtcatttcgaaaaaggttaggaatacggttagccatttgcctgcttttatatagttcantatgggattcacctttatgttgataagaaataaaagaaaatgccaataggatatcggcattttcttttgcgtttttatttgttaactgttaattgtccttgttcaaggatgctgtctttgacaacagatgttttcttgcctttgatgttcagcaggaagctcggcgcaaacgttgattgtttgtctgcgtagaatcctctgtttgtcatatagcttgtaatcacgacattgtttcctttcgcttgaggtacagcgaagtgtgagtaagtaaaggttacatcgttaggcggatcaagatccatttttaacacaaggccagttttgttcagcggcttgtatgggccagttaaagaattagaaacataaccaagcatgtaaatatcgttagacgtaatgccgtcaatcgtcatttttgatccgcgggagtcagtgaacaggtaccatttgccgttcattttaaagacgttcgcgcgttcaatttcatctgttactgtgttagatgcaatcagcggtttcatcacttttttcagtgtgtaatcatcgtttagctcaatcataccgagagcgccgtttgctaactcagccgtgcgttttttatcgctttgcagaagtttttgactttcttgacggaagaatgatgtgcttttgccatagtatgctttgttaaataaagattcttcgccttggtagccatcttcagttccagtgtttgcttcaaatactaagtatttgtggcctttatcttctacgtagtgaggatctctcagcgtatggttgtcgcctgagctgtagttgccttcatcgatgaactgctgtacattttgatacgtttttccgtcaccgtcaaagattgatttataatcctctacaccgttgatgttcaaagagctgtctgatgctgatacgttaacttgtgcagttgtcagtgtttgtttgccgtaatgtttaccggagaaatcagtgtagaataaacggatttttccgtcagatgtaaatgtggctgaacctgaccattcttgtgtttggtcttttaggatagaatcatttgcatcgaatttgtcgctgtctttaaagacgcggccagcgtttttccagctgtcaatagaagtttcgccgactttttgatagaacatgtaaatcgatgtgtcatccgcatttttaggatctccggctaatgcaaagacgatgtggtagccgtgatagtttgcgacagtgccgtcagcgttttgtaatggccagctgtcccaaacgtccaggccttttgcagaagagatatttttaattgtggacgaatcaaattcagaaacttgatatttttcatttttttgctgttcagggatttgcagcatatcatggcgtgtaatatgggaaatgccgtatgtttccttatatggcttttggttcgtttctttcgcaaacgcttgagttgcgcctcctgccagcagtgcggtagtaaaggttaatactgttgcttgttttgcaaactttttgatgttcatcgttcatgtctccttttttatgtactgtgttagcggtctgcttcttccagccctcctgtttgaagatggcaagttagttacgcacaataaaaaaagacctaaaatatgtaaggggtgacgccaaagtatacactttgccctttacacattttaggtcttgcctgctttatcagtaacaaacccgcgcgatttacttttcgacctcattctattagactctcgtttggattgcaactggtctattttcctcttttgtttgatagaaaatcataaaaggatttgcagactacgggcctaaagaactaaaaaatctatctgtttcttttcattctctgtattttttatagtttctgttgcatgggcataaagttgcctttttaatcacaattcagaaaatatcataatatctcatttcactaaataatagtgaacggcaggtatatgtgatgggttaaaaaggatcaccccagagtcccgctcagaagaactcgtcaagaaggcgatagaaggcgatgcgctgcgaatcgggagcggcgataccgtaaagcacgaggaagcggtcagcccattcgccgccaagctcttcagcaatatcacgggtagccaacgctatgtcctgatagcggtccgccacacccagccggccacagtcgatgaatccagaaaagcggccattttccaccatgatattcggcaagcaggcatcgccatgggtcacgacgagatcctcgccgtcgggcatccgcgccttgagcctggcgaacagttcggctggcgcgagcccctgatgctcttcgtccagatcatcctgatcgacaagaccggcttccatccgagtacgtgctcgctcgatgcgatgtttcgcttggtggtcgaatgggcaggtagccggatcaagcgtatgcagccgccgcattgcatcagccatgatggatactttctcggcaggagcaaggtgagatgacaggagatcctgccccggcacttcgcccaatagcagccagtcccttcccgcttcagtgacaacgtcgagacagctgcgcaaggaacgcccgtcgtggccagccacgatagccgcgctgcctcgtcttggagttcattcagggcaccggacaggtcggtcttgacaaaaagaaccgggcgcccctgcgctgacagccggaacacggcggcatcagagcagccgattgtctgttgtgcccagtcatagccgaatagcctctccacccaagcggccggagaacctgcgtgcaatccatcttgttcaatcatgcgaaacgatcctcatcctgtctcttgatcagatcttgatcccctgcgccatcagatccttggcggcaagaaagccatccagtttactttgcagggcttcccaaccttaccagagggcgccccagctggcaattccg

SEQ ID NO: 15 - DNA, 44 bp, Artificial Sequence
  primer 1
tcgagctcggtacccccgttcgtatgatcggttccgcacaggcc

SEQ ID NO: 16 - DNA, 31 bp, Artificial Sequence
  primer 2
gtgcagcaggcaaccacatcaaccgcccacg

SEQ ID NO: 17 - DNA, 31 bp, Artificial Sequence
  primer 3
cgtgggcggttgatgtggttgcctgctgcac

SEQ ID NO: 18 - DNA, 46 bp, Artificial Sequence
  primer 4
ctctagaggatccccgccgtaagcagcctctggtggaatggtcagc

SEQ ID NO: 19 - DNA, 31 bp, Artificial Sequence
  primer 5
gtgcagcaggcaactggatcaaccgcccacg

SEQ ID NO: 20 - DNA, 31 bp, Artificial Sequence
  primer 6
cgtgggcggttgatccagttgcctgctgcac

SEQ ID NO: 21 - DNA, 31 bp, Artificial Sequence
  primer 7
gtgcagcaggcaacggcatcaaccgcccacg

SEQ ID NO: 22 - DNA, 31 bp, Artificial Sequence
  primer 8
cgtgggcggttgatgccgttgcctgctgcac

SEQ ID NO: 23 - DNA, 29 bp, Artificial Sequence
  primer 9
ccgttcgtatgatcggttccgcacaggcc

SEQ ID NO: 24 - DNA, 31 bp, Artificial Sequence
  primer 10
gccgtaagcagcctctggtggaatggtcagc

SEQ ID NO: 25 - protein, 172 aa, Unknown
  IlvN AA
MANSDVTRHILSVLVQDVDGIISRVSGMFTRRAFNLVSLVSAKTETLGINRITVVVDADELNIEQITKQLNKLIPVLKVVRLDEETTIARAIMLVKVSADSTNRPQIVDAANIFRARVVDVAPDSVVIESTGTPGKLRALLDVMEPFGIRELIQSGQIALNRGPKTMAPAKI

SEQ ID NO: 26 - DNA, 520 bp, Unknown
  IlvN NT
atggctaattctgacgtcacccgccacatcctgtccgtactcgttcaggacgtagacggaatcatttcccgcgtatcaggtatgttcacccgacgcgcattcaacctcgtgtccctcgtgtctgcaaagaccgaaacactcggcatcaaccgcatcacggttgttgtcgacgccgacgagctcaacattgagcagatcaccaagcagctcaacaagctgatccccgtgctcaaagtcgtgcgacttgatgaagagaccaccatcgcccgcgcaatcatgctggttaaggtctctgcggatagcaccaaccgtccgcagatcgtcgacgccgcgaacatcttccgcgcccgagtcgtcgacgtggctccagactctgtggttattgaatccacaggcaccccaggcaagctccgcgcactgcttgatgtgatggaaccattcggaatccgcgaactgatccaatccggacagattgcactcaaccgcggtccgaagaccatggctccggccaagatctaaa

SEQ ID NO: 27 - protein, 172 aa, Artificial Sequence
  IlvN A42V AA
MANSDVTRHILSVLVQDVDGIISRVSGMFTRRAFNLVSLVSVKTETLGINRITVVVDADELNIEQITKQLNKLIPVLKVVRLDEETTIARAIMLVKVSADSTNRPQIVDAANIFRARVVDVAPDSVVIESTGTPGKLRALLDVMEPFGIRELIQSGQIALNRGPKTMAPAKI

SEQ ID NO: 28 - DNA, 519 bp, Artificial Sequence
  IlvN A42V NT
atggctaattctgacgtcacccgccacatcctgtccgtactcgttcaggacgtagacggaatcatttcccgcgtatcaggtatgttcacccgacgcgcattcaacctcgtgtccctcgtgtctgtaaagaccgaaacactcggcatcaaccgcatcacggttgttgtcgacgccgacgagctcaacattgagcagatcaccaagcagctcaacaagctgatccccgtgctcaaagtcgtgcgacttgatgaagagaccaccatcgcccgcgcaatcatgctggttaaggtctctgcggatagcaccaaccgtccgcagatcgtcgacgccgcgaacatcttccgcgcccgagtcgtcgacgtggctccagactctgtggttattgaatccacaggcaccccaggcaagctccgcgcactgcttgatgtgatggaaccattcggaatccgcgaactgatccaatccggacagattgcactcaaccgcggtccgaagaccatggctccggccaagatctaa

SEQ ID NO: 29 - DNA, 33 bp, Artificial Sequence
  primer 11
tcgagctcggtacccccgcgtcaccaaagcgga

SEQ ID NO: 30 - DNA, 30 bp, Artificial Sequence
  primer 12
gtccctcgtgtctgtaaagaccgaaacact

SEQ ID NO: 31 - DNA, 30 bp, Artificial Sequence
  primer 13
agtgtttcggtctttacagacacgagggac

SEQ ID NO: 32 - DNA, 35 bp, Artificial Sequence
  primer 14
ctctagaggatccccttagatcttggccggagcca

SEQ ID NO: 33 - DNA, 18 bp, Artificial Sequence
  primer 15
ccgcgtcaccaaagcgga

SEQ ID NO: 34 - DNA, 20 bp, Artificial Sequence
  primer 16
ttagatcttggccggagcca

SEQ ID NO: 35 - protein, 418 aa, Unknown
  YjeH AA
MSGLKQELGLAQGIGLLSTSLLGTGVFAVPALAALVAGNNSLWAWPVLIILVFPIAIVFAILGRHYPSAGGVAHFVGMAFGSRLERVTGWLFLSVIPVGLPAALQIAAGFGQAMFGWHSWQLLLAELGTLALVWYIGTRGASSSANLQTVIAGLIVALIVAIWWAGDIKPANIPFPAPGNIELTGLFAALSVMFWCFVGLEAFAHLASEFKNPERDFPRALMIGLLLAGLVYWGCTVVVLHFDAYGEKMAAAASLPKIVVQLFGVGALWIACVIGYLACFASLNIYIQSFARLVWSQAQHNPDHYLARLSSRHIPNNALNAVLGCCVVSTLVIHALEINLDALIIYANGIFIMIYLLCMLAGCKLLQGRYRLLAVVGGLLCVLLLAMVGWKSLYALIMLAGLWLLLPKRKTPENGITT

SEQ ID NO: 36 - DNA, 1257 bp, Unknown
  YjeH NT
atgagtggactcaaacaagaactggggctggcccagggcattggcctgctatcgacgtcattattaggcactggcgtgtttgccgttcctgcgttagctgcgctggtagcgggcaataacagcctgtgggcgtggcccgttttgattatcttagtgttcccgattgcgattgtgtttgcgattctgggtcgccactatcccagcgcaggcggcgtcgcgcacttcgtcggtatggcgtttggttcgcggcttgagcgagtcaccggctggctgtttttatcggtcattcccgtgggtttgcctgccgcactacaaattgccgccgggttcggccaggcgatgtttggctggcatagctggcaactgttgttggcagaactcggtacgctggcgctggtgtggtatatcggtactcgcggtgccagttccagtgctaatctacaaaccgttattgccggacttatcgtcgcgctgattgtcgctatctggtgggcgggcgatatcaaacctgcgaatatcccctttccggcacctggtaatatcgaacttaccgggttatttgctgcgttatcagtgatgttctggtgttttgtcggtctggaggcatttgcccatctcgcctcggaatttaaaaatccagagcgtgattttcctcgtgctttgatgattggtctgctgctggcaggattagtctactggggctgtacggtagtcgtcttacacttcgacgcctatggtgaaaaaatggcggcggcagcatcgcttccaaaaattgtagtgcagttgttcggtgtaggagcgttatggattgcctgcgtgattggctatctggcctgctttgccagtctcaacatttatatacagagcttcgcccgcctggtctggtcgcaggcgcaacataatcctgaccactacctggcacgcctctcttctcgccatatcccgaataatgccctcaatgcggtgctcggctgctgtgtggtgagcactttggtgattcatgctttagagatcaatctggacgctcttattatttatgccaatggcatctttattatgatttatctgttatgcatgctggcaggctgtaaattattgcaaggacgttatcgactactggcggtggttggcgggctgttatgcgttctgttactggcaatggtcggctggaaaagtctctatgcgctgatcatgctggcggggttatggctgttgctgccaaaacgaaaaacgccggaaaatggcataaccacataa

SEQ ID NO: 37 - protein, 88 aa, Unknown
  NCgl2335 AA
MAYTFDHVVAWRWCTKEDAYNYTHLFDQLQPPLIVTTDGQKRRTQSHHHDLADNENPTLPRPRQTQRPKTRHPKTRAELAEKHSGVSP

SEQ ID NO: 38 - DNA, 267 bp, Unknown
  NCgl2335 NT
gtggcctacaccttcgaccacgtcgtcgcctggcgctggtgcaccaaagaagacgcctacaactacacccacctcttcgatcaactccaaccacccttaatcgtgaccaccgacggacaaaaaaggcgcactcaaagccatcaccacgacctggccgacaacgaaaatccaacgctgcctcgtccacgtcaaacgcaacgtccaaaaacacgtcaccctaagacccgtgctgagctcgccgaaaagcactccggggtctctccttga

SEQ ID NO: 39 - DNA, 39 bp, Artificial Sequence
  Tn_5 F
tgaattcgagctcggtaccccaccgacgcgcatctgcct

SEQ ID NO: 40 - DNA, 50 bp, Artificial Sequence
  Tn_5 R
ggtgtggtgactttcagcagttcccgggggggaggaggcatgtggtgttg

SEQ ID NO: 41 - DNA, 50 bp, Artificial Sequence
  Tn_3 F
caacaccacatgcctcctcccccccgggaactgctgaaagtcaccacacc

SEQ ID NO: 42 - DNA, 42 bp, Artificial Sequence
  Tn_3 R
gtcgactctagaggatccccctcccaaaccattgaggaatgg

SEQ ID NO: 43 - DNA, 39 bp, Artificial Sequence
  CJ7_yjeH F
acaccacatgcctcctccccagaaacatcccagcgctac

SEQ ID NO: 44 - DNA, 43 bp, Artificial Sequence
  CJ7_yjeH R
agttcttgtttgagtccactcatagtgtttcctttcgttgggt

SEQ ID NO: 45 - DNA, 44 bp, Artificial Sequence
  yjeH F
acccaacgaaaggaaacactatgagtggactcaaacaagaactg

SEQ ID NO: 46 - DNA, 44 bp, Artificial Sequence
  yjeH R
gactttcagcagttcccgggttatgtggttatgccattttccgg

SEQ ID NO: 47 - protein, 418 aa, Artificial Sequence
  yjeH F351L AA
MSGLKQELGLAQGIGLLSTSLLGTGVFAVPALAALVAGNNSLWAWPVLIILVFPIAIVFAILGRHYPSAGGVAHFVGMAFGSRLERVTGWLFLSVIPVGLPAALQIAAGFGQAMFGWHSWQLLLAELGTLALVWYIGTRGASSSANLQTVIAGLIVALIVAIWWAGDIKPANIPFPAPGNIELTGLFAALSVMFWCFVGLEAFAHLASEFKNPERDFPRALMIGLLLAGLVYWGCTVVVLHFDAYGEKMAAAASLPKIVVQLFGVGALWIACVIGYLACFASLNIYIQSFARLVWSQAQHNPDHYLARLSSRHIPNNALNAVLGCCVVSTLVIHALEINLDALIIYANGILIMIYLLCMLAGCKLLQGRYRLLAVVGGLLCVLLLAMVGWKSLYALIMLAGLWLLLPKRKTPENGITT

SEQ ID NO: 48 - DNA, 1257 bp, Artificial Sequence
  yjeH F351L NT
atgagtggactcaaacaagaactggggctggcccagggcattggcctgctatcgacgtcattattaggcactggcgtgtttgccgttcctgcgttagctgcgctggtagcgggcaataacagcctgtgggcgtggcccgttttgattatcttagtgttcccgattgcgattgtgtttgcgattctgggtcgccactatcccagcgcaggcggcgtcgcgcacttcgtcggtatggcgtttggttcgcggcttgagcgagtcaccggctggctgaatttatcggtcattcccgtgggtttgcctgccgcactacaaattgccgccgggttcggccaggcgatgtttggctggcatagctggcaactgttgttggcagaactcggtacgctggcgctggtgtggtatatcggtactcgcggtgccagttccagtgctaatctacaaaccgttattgccggacttatcgtcgcgctgattgtcgctatctggtgggcgggcgatatcaaacctgcgaatatcccctttccggcacctggtaatatcgaacttaccgggttatttgctgcgttatcagtgatgttctggtgttttgtcggtctggaggcatttgcccatctcgcctcggaatttaaaaatccagagcgtgattttcctcgtgctttgatgattggtctgctgctggcaggattagtctactggggctgtacggtagtcgtcttacacttcgacgcctatggtgaaaaaatggcggcggcagcatcgcttccaaaaattgtagtgcagttgttcggtgtaggagcgttatggattgcctgcgtgattggctatctggcctgctttgccagtctcaacatttatatacagagcttcgcccgcctggtctggtcgcaggcgcaacataatcctgaccactacctggcacgcctctcttctcgccatatcccgaataatgccctcaatgcggtgctcggctgctgtgtggtgagcactttggtgattcatgctttagagatcaatctggacgctcttattatttatgccaatggcatccttattatgatttatctgttatgcatgctggcaggctgtaaattattgcaaggacgttatcgactactggcggtggttggcgggctgttatgcgttctgttactggcaatggtcggctggaaaagtctctatgcgctgatcatgctggcggggttatggctgttgctgccaaaacgaaaaacgccggaaaatggcataaccacataa

SEQ ID NO: 49 - DNA, 23 bp, Artificial Sequence
  F351L F
caatggcatccttattatgattt

SEQ ID NO: 50 - DNA, 23 bp, Artificial Sequence
  F351L R
aaatcataataaggatgccattg

SEQ ID NO: 51 - protein, 127 aa, Artificial Sequence
  General formula 1(GltA 289~415)
  MISC_FEATURE (1): Xaa is N or S.
  MISC_FEATURE (9): Xaa is A or E.
  MISC_FEATURE (73): Xaa is Y or C.
XNHGGDATXFMNKVKNKEDGVRLMGFGHRVYKNYDPRAAIVKETAHEILEHLGGDDLLDLAIKLEEIALADDXFISRKLYPNVDFYTGLIYRAMGFPTDFFTVLFAIGRLPGWIAHYREQLGAAGNH